European Patent Application EP 4 248 995 A1, published September 27, 2023. Title: USE OF ANTI-OX40 ANTIBODY IN TREATMENT OF TUMOR OR CANCER. Applicant: Bio-Thera Solutions, Ltd. Application EP21893986.6. The sequence listing filed with the application follows.

SEQUENCE LISTING (12 sequences)

SEQ ID NO: 1 - protein, 5 aa, Artificial Sequence
  synthetic construct
SYGMH

SEQ ID NO: 2 - protein, 17 aa, Artificial Sequence
  synthetic construct
VIWEDGSNQYYADSVKG

SEQ ID NO: 3 - protein, 13 aa, Artificial Sequence
  synthetic construct
DNQDTSPDVGIDY

SEQ ID NO: 4 - protein, 11 aa, Artificial Sequence
  synthetic construct
RASQNISPFLN

SEQ ID NO: 5 - protein, 7 aa, Artificial Sequence
  synthetic construct
AAVGLQS

SEQ ID NO: 6 - protein, 9 aa, Artificial Sequence
  synthetic construct
QQYTDYPLT

SEQ ID NO: 7 - protein, 122 aa, Artificial Sequence
  synthetic construct
QVQLVESGGGVVQPGESLRLSCAASGFTFSSYGMHWVRQAPGKGLEWVAVIWEDGSNQYYADSVKGRFTISRDNSKNTLYLQMNSLRAEDTAVYYCAKDNQDTSPDVGIDYWGQGTLVTVSS

SEQ ID NO: 8 - protein, 107 aa, Artificial Sequence
  synthetic construct
DIQMTQSPSSLSASVGDRVTITCRASQNISPFLNWYQQKPGKAPKLLIYAAVGLQSGVPSRFSGSGSGTDFTLTISSLQPEDFATYYCQQYTDYPLTFGGGTKVEIK

SEQ ID NO: 9 - protein, 452 aa, Artificial Sequence
  synthetic construct
QVQLVESGGGVVQPGESLRLSCAASGFTFSSYGMHWVRQAPGKGLEWVAVIWEDGSNQYYADSVKGRFTISRDNSKNTLYLQMNSLRAEDTAVYYCAKDNQDTSPDVGIDYWGQGTLVTVSSASTKGPSVFPLAPSSKSTSGGTAALGCLVKDYFPEPVTVSWNSGALTSGVHTFPAVLQSSGLYSLSSVVTVPSSSLGTQTYICNVNHKPSNTKVDKKVEPKSCDKTHTCPPCPAPELLGGPSVFLFPPKPKDTLMISRTPEVTCVVVDVSHEDPEVKFNWYVDGVEVHNAKTKPREEQYNSTYRVVSVLTVLHQDWLNGKEYKCKVSNKALPAPIEKTISKAKGQPREPQVYTLPPSRDELTKNQVSLTCLVKGFYPSDIAVEWESNGQPENNYKTTPPVLDSDGSFFLYSKLTVDKSRWQQGNVFSCSVMHEALHNHYTQKSLSLSPGK

SEQ ID NO: 10 - protein, 214 aa, Artificial Sequence
  synthetic construct
DIQMTQSPSSLSASVGDRVTITCRASQNISPFLNWYQQKPGKAPKLLIYAAVGLQSGVPSRFSGSGSGTDFTLTISSLQPEDFATYYCQQYTDYPLTFGGGTKVEIKRTVAAPSVFIFPPSDEQLKSGTASVVCLLNNFYPREAKVQWKVDNALQSGNSQESVTEQDSKDSTYSLSSTLTLSKADYEKHKVYACEVTHQGLSSPVTKSFNRGEC

SEQ ID NO: 11 - DNA, 1413 bp, Artificial Sequence
  synthetic construct
atggagttcggactgagctgggtgtttctggtggccattctgaaaggcgtgcagtgccaagtgcagctggtggagagcggaggaggagtggtgcaacccggcgagtccctcagactgagctgtgccgccagcggcttcaccttcagctcctacggcatgcactgggtgagacaagcccccggcaaaggactggagtgggtggccgtgatctgggaggatggctccaaccagtactatgccgacagcgtgaagggaagattcaccatctctagagacaactccaagaacacactgtatctgcagatgaactctctgagggccgaggacaccgccgtgtactactgcgccaaggacaaccaagacaccagccccgacgtgggcatcgattattggggccagggtaccctggttaccgttagcagcgcgagcaccaaaggcccgagcgtgtttccgctggccccgagcagcaaaagcaccagcggtggcaccgcagcgctgggttgcctggtgaaagattatttcccggaaccggtgacggtgtcgtggaactcaggcgccctgaccagcggcgtgcacaccttcccggctgtcctacagtcctcaggactctactccctcagcagcgtggtgaccgtgccctccagcagcttgggcacccagacctacatctgcaacgtgaatcacaagcccagcaacaccaaggtggacaagaaagttgagcccaaatcttgtgacaaaactcacacatgcccaccgtgcccagcacctgaactcctggggggaccgtcagtcttcctcttccccccaaaacccaaggacaccctcatgatctcccggacccctgaggtcacatgcgtggtggtggacgtgagccacgaagaccctgaggtcaagttcaactggtacgtggacggcgtggaggtgcataatgccaagacaaagccgcgggaggagcagtacaacagcacgtaccgtgtggtcagcgtcctcaccgtcctgcaccaggactggctgaatggcaaggagtacaagtgcaaggtctccaacaaagccctcccagcccccatcgagaaaaccatctccaaagccaaagggcagccccgagaaccacaggtgtacaccctgcccccatcccgggatgagctgaccaagaaccaggtcagcctgacctgcctggtcaaaggcttctatcccagcgacatcgccgtggagtgggagagcaatgggcagccggagaacaactacaagaccacgcctcccgtgctggactccgacggctccttcttcctctacagcaagctcaccgtggacaagagcaggtggcagcaggggaacgtcttctcatgctccgtgatgcatgaggctctgcacaaccactacacgcagaagagcctctccctgtctccgggtaaa

SEQ ID NO: 12 - DNA, 708 bp, Artificial Sequence
  synthetic construct
atggacatgagagtgctggctcagctgctgggactgctgctgctgtgctttcccggcgccagatgcgacatccagatgacccagagccctagctctctgtccgctagcgtgggagatagagtgaccatcacatgcagagccagccagaacatctccccctttctgaattggtatcagcagaagcccggcaaggcccctaagctgctgatctatgccgctgtgggactgcagagcggagtgccttccagattctccggcagcggcagcggaaccgacttcacactgaccatcagctctctgcagcccgaggacttcgccacctactactgccagcagtataccgactaccctctgaccttcggaggcggcaccaaggtggagatcaagcgtacggtggctgcaccatctgtcttcatcttcccgccatctgatgagcagttgaaatctggaactgcctctgttgtgtgcctgctgaataacttctatcccagagaggccaaagtacagtggaaggtggataacgccctccaatcgggtaactcccaggagagtgtcacagagcaggacagcaaggacagcacctacagcctcagcagcaccctgacgctgagcaaagcagactacgagaaacacaaagtctacgcctgcgaagtcacccatcagggcctgagctcgcccgtcacaaagagcttcaacaggggagagtgt